European Patent Application EP 4 187 246 A1, published May 31, 2023. Title: Method for Aiding in Diagnosis of Inflammatory Bowel Disease. Applicant: FUJIFILM Wako Pure Chemical Corporation Osaka University. The sequence listing filed with the application follows.

SEQUENCE LISTING (5 sequences)

SEQ ID NO: 1 - protein, 6 aa, Homo sapiens
QCKNYY

SEQ ID NO: 2 - protein, 102 aa, Homo sapiens
  SIGNAL (1)..(18)
MSALGAVIALLLWGQLFAVDSGNDVTDIADDGCPKPPEIAHGYVEHSVRYQCKNYYKLRTEGDGVYTLNDKKQWINKAVGDKLPECEAVCGKPKNPANPVQR

SEQ ID NO: 3 - protein, 161 aa, Homo sapiens
  SIGNAL (1)..(18)
MSALGAVIALLLWGQLFAVDSGNDVTDIADDGCPKPPEIAHGYVEHSVRYQCKNYYKLRTEGDGVYTLNDKKQWINKAVGDKLPECEADDGCPKPPEIAHGYVEHSVRYQCKNYYKLRTEGDGVYTLNNEKQWINKAVGDKLPECEAVCGKPKNPANPVQR

SEQ ID NO: 4 - DNA, 42 bp, Artificial Sequence
  Oligonucleotide primer
ccaagaatccggcaaacccagtgcagcagatcctgggtggac

SEQ ID NO: 5 - DNA, 43 bp, Artificial Sequence
  Oligonucleotide primer
ggcatccaggtgtccacccaggatctgctgcactgggtttgcc